European Patent Application EP 4 649 947 A2, published November 19, 2025. Title: Methods for treating against viruses. Applicant: Howard University. Application EP 25188917.6, filed April 27, 2020. The sequence listing filed with the application follows.

SEQUENCE LISTING (12 sequences)

SEQ ID NO: 1 - DNA, 17 bp, synthetic construct
  misc_feature 1..17: note = primer for HSV-1 ICP0 - forward
  source 1..17: mol_type = other DNA
ctgcgctgcgacacctt

SEQ ID NO: 2 - DNA, 22 bp, synthetic construct
  misc_feature 1..22: note = primer for HSV-1 ICP0 - reverse
  source 1..22: mol_type = other DNA
caattgcatccaggttttcatg

SEQ ID NO: 3 - DNA, 21 bp, synthetic construct
  misc_feature 1..21: note = primer for beta-actin - forward
  source 1..21: mol_type = other DNA
ggttccgatgccctgaggctc

SEQ ID NO: 4 - DNA, 21 bp, synthetic construct
  misc_feature 1..21: note = primer for beta-actin - reverse
  source 1..21: mol_type = other DNA
acttgcggtgcacgatggagg

SEQ ID NO: 5 - protein, 14 aa, synthetic construct
  REGION 1..14: note = Synthetic peptide sequence
FSPNRYWLCAATEN

SEQ ID NO: 6 - RNA, 39 nt, synthetic construct
  misc_feature 1..39: note = 13462 to 13490 bp of SARS-CoV-2 Wuhan-Hu-1
  source 1..39: mol_type = other RNA
tttaaacgggtttgcggtgtaagtgcagcccgtcttaca

SEQ ID NO: 7 - protein, 10 aa, synthetic construct
  REGION 1..10: note = Annexin A2 fragment 1
TNQELQEINR

SEQ ID NO: 8 - protein, 14 aa, synthetic construct
  REGION 1..14: note = Annexin A2 fragment 2
GVDEVTIVNILTNR

SEQ ID NO: 9 - protein, 10 aa, synthetic construct
  REGION 1..10: note = Annexin A2 fragment 3
DALNIETAIK

SEQ ID NO: 10 - protein, 14 aa, synthetic construct
  MOD_RES 6: note = phosphotyrosine
FSPNRYWLCAATEH

SEQ ID NO: 11 - RNA, 13 nt, Human coronavirus HKU1
  source 1..13: mol_type = other RNA
atttattgtttgg

SEQ ID NO: 12 - RNA, 13 nt, coronavirus mhv
  source 1..13: mol_type = other RNA
ttttattcttttt